European Patent Application EP 4 299 587 A1, published January 3, 2024. Title: Method of detecting malignant pancreatic cystic tumors, antibodies and detection kit for malignant pancreatic cystic tumors. Applicant: TORAY Industries, Inc. National Cancer Center. The sequence listing filed with the application follows.

SEQUENCE LISTING (50 sequences)

SEQ ID NO: 1 - protein, 76 aa, Homo sapiens
QAKEPCVESLVSQYFQTVTDYGKDLMEKVKSPELQAEAKSYFEKSKEQLTPLIKKAGTELVNFLSYFVELGTQPAT

SEQ ID NO: 2 - protein, 77 aa, Homo sapiens
QAKEPCVESLVSQYFQTVTDYGKDLMEKVKSPELQAEAKSYFEKSKEQLTPLIKKAGTELVNFLSYFVELGTQPATQ

SEQ ID NO: 3 - protein, 75 aa, Homo sapiens
QAKEPCVESLVSQYFQTVTDYGKDLMEKVKSPELQAEAKSYFEKSKEQLTPLIKKAGTELVNFLSYFVELGTQPA

SEQ ID NO: 4 - protein, 10 aa, Artificial Sequence
  antibody
GYTFTNYWMH

SEQ ID NO: 5 - protein, 17 aa, Artificial Sequence
  antibody
NIYPGSGNTNYNEKFKS

SEQ ID NO: 6 - protein, 10 aa, Artificial Sequence
  antibody
RYGYVDWFAY

SEQ ID NO: 7 - protein, 16 aa, Artificial Sequence
  antibody
RSSKSLLYKDGKTYLN

SEQ ID NO: 8 - protein, 7 aa, Artificial Sequence
  antibody
LMSTRAS

SEQ ID NO: 9 - protein, 9 aa, Artificial Sequence
  antibody
QQLVEYPLT

SEQ ID NO: 10 - protein, 5 aa, Artificial Sequence
  antibody
NYGMN

SEQ ID NO: 11 - protein, 17 aa, Artificial Sequence
  antibody
WKNTYTGESTYADDFKG

SEQ ID NO: 12 - protein, 11 aa, Artificial Sequence
  antibody
RDGSKYKIFDY

SEQ ID NO: 13 - protein, 12 aa, Artificial Sequence
  antibody
RASSSLSSSYLH

SEQ ID NO: 14 - protein, 7 aa, Artificial Sequence
  antibody
STSNLAS

SEQ ID NO: 15 - protein, 9 aa, Artificial Sequence
  antibody
QQFSVFPLT

SEQ ID NO: 16 - protein, 10 aa, Artificial Sequence
  antibody
GYTFTSYWMH

SEQ ID NO: 17 - protein, 17 aa, Artificial Sequence
  antibody
FINPSTGYTENNQRFND

SEQ ID NO: 18 - protein, 10 aa, Artificial Sequence
  antibody
RPYNPYAMDY

SEQ ID NO: 19 - protein, 11 aa, Artificial Sequence
  antibody
RASQDTSNYLN

SEQ ID NO: 20 - protein, 7 aa, Artificial Sequence
  antibody
YTSRLHS

SEQ ID NO: 21 - protein, 9 aa, Artificial Sequence
  antibody
QQGNTLPYT

SEQ ID NO: 22 - protein, 10 aa, Artificial Sequence
  antibody
GYTFTSYWMH

SEQ ID NO: 23 - protein, 17 aa, Artificial Sequence
  antibody
FINPSTGYTENNQNFKE

SEQ ID NO: 24 - protein, 10 aa, Artificial Sequence
  antibody
RTYNPYGMDY

SEQ ID NO: 25 - protein, 11 aa, Artificial Sequence
  antibody
RASQDISNYLN

SEQ ID NO: 26 - protein, 7 aa, Artificial Sequence
  antibody
YTSRLQS

SEQ ID NO: 27 - protein, 9 aa, Artificial Sequence
  antibody
QQGNTLPYT

SEQ ID NO: 28 - protein, 16 aa, Homo sapiens
VNFLSYFVELGTQPAT

SEQ ID NO: 29 - protein, 17 aa, Homo sapiens
VNFLSYFVELGTQPATQ

SEQ ID NO: 30 - protein, 6 aa, Homo sapiens
GTQPAT

SEQ ID NO: 31 - protein, 6 aa, Homo sapiens
TQPATQ

SEQ ID NO: 32 - protein, 6 aa, Homo sapiens
LGTQPA

SEQ ID NO: 33 - protein, 5 aa, Artificial Sequence
  antibody
NYGMN

SEQ ID NO: 34 - protein, 17 aa, Artificial Sequence
  antibody
WINTYTGEPTYTNDFKG

SEQ ID NO: 35 - protein, 11 aa, Artificial Sequence
  antibody
GRGYDEGWFAY

SEQ ID NO: 36 - protein, 12 aa, Artificial Sequence
  antibody
TASSSMSSTYLH

SEQ ID NO: 37 - protein, 7 aa, Artificial Sequence
  antibody
RTSTLAS

SEQ ID NO: 38 - protein, 9 aa, Artificial Sequence
  antibody
QQGSRKPYT

SEQ ID NO: 39 - protein, 5 aa, Artificial Sequence
  antibody
NFGMN

SEQ ID NO: 40 - protein, 17 aa, Artificial Sequence
  antibody
WINTYTGEPAYTSDFKG

SEQ ID NO: 41 - protein, 11 aa, Artificial Sequence
  antibody
GRGYDEGWFAY

SEQ ID NO: 42 - protein, 12 aa, Artificial Sequence
  antibody
TASSSMSSTYLH

SEQ ID NO: 43 - protein, 7 aa, Artificial Sequence
  antibody
RTSTLAS

SEQ ID NO: 44 - protein, 9 aa, Artificial Sequence
  antibody
QQGSRKPYT

SEQ ID NO: 45 - protein, 5 aa, Artificial Sequence
  antibody
NYGMN

SEQ ID NO: 46 - protein, 17 aa, Artificial Sequence
  antibody
WINTYTGEPTYVDDFKG

SEQ ID NO: 47 - protein, 11 aa, Artificial Sequence
  antibody
GRGYDEGWLVY

SEQ ID NO: 48 - protein, 12 aa, Artificial Sequence
  antibody
SSSSSMSSTYLH

SEQ ID NO: 49 - protein, 7 aa, Artificial Sequence
  antibody
RTSNLAS

SEQ ID NO: 50 - protein, 9 aa, Artificial Sequence
  antibody
QQGSRKPFT